European Patent Specification EP 3 658 610 B1, published October 25, 2023. Title: GH5 AND GH30 IN WET MILLING. Applicant: Novozymes A/S. The sequence listing filed with the application follows.

SEQUENCE LISTING (12 sequences)

SEQ ID NO: 1 - protein, 655 aa, Ruminiclostridium thermocellum
MKKPLGKIVASTALLISVAFSSSIASAHHHHHHPRADPQRGRPYLNSARTTFVGDNGQPLRGPYISTEWTSAAPYDQIARIKNLGFNAVHHYAECFDINYPNAGSKSPGYAATEIDKVVERTRELGLYLVMTIGNGANNGNHNTRYAKDFWSFYSSRYANETHVLYEIHNEPVAWGPPYSSTTATPTGAVEMNVDVYKTIRANAPKTPVLIFSYSVFGGTGGTTEALKDIQAFNSAVFGKQDAVWTNEAVAFHGYAGWEATSTAVDGLLKAGYPCFMTEYAGGAWGSGTGGFDIQLTSELERMGVSWLTFQYIPPSGVSDDVTKPEYFSALVENAGLSWKPDYGNWPAARGVHGNGGLPRKTSTWVNNFLTGTTRIEAEDFDWGGNDVSFYDKDSENKGAQYRLDEAVDIETTKDADGGYNVGWIEDGEWLEYTIWVQHPGYYNLALRVANNSGGSVQVNFGNQDKTGTWVLPVTGGVQTWKTDTRQVFLGSGRQKLRINALSGGFNLNWIELSPVSTGPIADGTYKFLNRANTMTLQEVTSNNSIVTSTYKGTADQHWKIQHIGGGQYRISSAGRGWNWNWWMGFGTVGWWGTGSGTCFIIRPTGDGYYRFVLVNDGTNLEISNNDSSKIEGKAYHEGANQQWAIQLPSAPVFP

SEQ ID NO: 2 - protein, 555 aa, Paenibacillus sp-18054
HHHHHHPRLTVPPGAPAEAWSGMPTPKLHVSGNQLVNANGQPVLLSGWHQPSGSYWTYQSSSYYLDRNGGNRHAANLAYLKDITDTFTDTSPKYGNNHGWYMNQVRLFIDREDMGDVAEGTYNFAGLQAVTQNVIIPYINYARTKGLYVTLGLDFTLKDNQATTQANLDKFNQIWSYLASRPEIRSADNVMFEIINEPVLSYADGRWGGHPSDPHFIAFWNDLRSFQNSIISSIRAQGADNVIWAAGLGWDQYYQLCASHPLTDPLNNVGYAVHWYPGYGAGDNYSVLQQQWDTNIKPCADNYPINITETTWFKRLPGDSDYWNLFNGSSEGFGKNTKAIFTAAGNASIAVHMNGFLLAPGARSSFADPTAGLLYDGNTARDGMARFIFEWYYERAQFLPWNGIWNGLFTGSTYKFVNRATGKNMDVPGGQNNNNLQLNQWTDNGATAQRWVVDDMGTFNNIYRMKSVSSSDGKVMDVRNGTKNNGEAIQLMQDFSNTAQRFRIIRLSNGYWSIINVNSNKAVEVAGGASHDGALLQQNMYRGDHHQQWQLVQIQ

SEQ ID NO: 3 - protein, 585 aa, Chryseobacterium sp-10696
MKKPLGKIVASTALLISVAFSSSIASAHHHHHHPRDEKNLLEDPDSNLSAGASARALAATPMLHVGGRYLKDPCDNNVVLHGVAITPSPWFNGCQYGANSGYCTWDNYNVQGALNYNKAVMNKLTSAADGWYLNYIRLHIDPYWTNDPGPAIPENDISRFNYNRLVTYTDQVIIPLINHARSLGMYVILRPPGVCPNRIAVNDAYHSYLKTVWTFLSQHPGLKNADNVMFELANEPVEILGTNGTWGSTGNEHFAALKNFFQPLVNIIRNNGANNVCWIPGTGWQSHYQGYVNNQITGGNIGYAVHIYPAYWGGLSNYQAFQNAWNINVKPIADIAPIAITETDWAPQGYGTFGIGTTGTAGGSGFGANLKYIVDQSGNVSWNVLAPDNLLHKGDPNAGTAYNNDWEACAAPVKQWFQQYASSNYPVGNCNTTSSLVNNGIYEIEFQTDANKVVDLKSGEDANGAVLRPWTRNGAAAQRWVAIDAGNGYWRFVSKASATNRCIDLASNSNTLGTSIRLWQNYGNDAQAWQVVAVSNGYYKILSKVDPTRGWDIPNCTMDGNSNLHLWDYYGTSCQLFKFKYIGMN

SEQ ID NO: 4 - protein, 391 aa, Bacillus subtilis
AASDVTVNVSAEKQVIRGFGGMNHPAWAGDLTAAQRETAFGNGQNQLGFSILRIHVDENRNNWYKEVETAKSAVKHGAIVFASPWNPPSDMVETFNRNGDTSAKRLKYNKYAAYAQHLNDFVTFMKNNGVNLYAISVQNEPDYAHEWTWWTPQEILRFMRENAGSINARVIAPESFQYLKNLSDPILNDPQALANMDILGTHLYGTQVSQFPYPLFKQKGAGKDLWMTEVYYPNSDTNSADRWPEALDVSQHIHNAMVEGDFQAYVWWYIRRSYGPMKEDGTISKRGYNMAHFSKFVRPGYVRIDATKNPNANVYVSAYKGDNKVVIVAINKSNTGVNQNFVLQNGSASNVSRWITSSSSNLQPGTNLTVSGNHFWAHLPAQSVTTFVVNR

SEQ ID NO: 5 - protein, 417 aa, Bacillus subtilis
MKKPLGKIVASTALLISVAFSSSIASAASDVTVNVSAEKQVIRGFGGMNWPAWAGDLTAAQRETAFGNGQNQLGFSILRIHVDENRNNWYKEVETAKSALKLGAIVFASPWNPPSDMVETFNRNGDTSAKRLKYNKYAAYAQHLNDFVTFMKNNGVNLYAISVQNEPDYAHEWTWWTPQEMLRFMRENAGSINARVIAPESFQYLKNLSDPILNDPQALANMDILGTHLYGTQLSQFPYPLFKQKGAGKDLWMTEVYYPNSDTNSADRWPEALDVSQHIHNAMVEGDFQAYVWWYIRRSYGPMKEDGTISKRGYNMAHFSKFVRPGYVRIDATKNPNANVYVSAYKGDNKVVIVAINKSNTGVNQNFVLQNGSASNVSRWITSSSSNLQPGTNLTVSGNHFWAHLPAQSVTTFVVNR

SEQ ID NO: 6 - protein, 417 aa, Bacillus subtilis
MKKPLGKIVASTALLISVAFSSSIASAASDVTVNVSAEKQVIRGFGGMNWPAWAGDLTAAQRETAFGNGQNQLGFSILRIHVDENRNNWYKEVETAKSAVLLGAIVFASPWNPPSDMVETFNRNGDTSAKRLKYNKYAAYAQHLNDFVTFMKNNGVNLYAISVQNEPDYAHEWTWWTPQEMLRFMRENAGSINARVIAPESFQYLKNLSDPILNDPQALANMDILGTHLYGTQLSQFPYPLFKQKGAGKDLWMTEVYYPNSDTNSADRWPEALDVSQHIHNAMVEGDFQAYVWWYIRRSYGPMKEDGTISKRGYNMAHFSKFVRPGYVRIDATKNPNANVYVSAYKGDNKVVIVAINKSNTGVNQNFVLQNGSASNVSRWITSSSSNLQPGTNLTVSGNHFWAHLPAQSVTTFVVNR

SEQ ID NO: 7 - protein, 417 aa, Bacillus subtilis
MKKPLGKIVASTALLISVAFSSSIASAASDVTVNVSAEKQVIRGFGGMNHPAWAGDLTAAQRETAFGNGQNQLGFSILRIHVDENRNNWYKEVETAKSAVKHGAIVFASPWNPPSDMVETFNRNGDTSAKRLKYNKYAAYAQHLNDFVTFMKNNGVNLYAISVQNEPDYAHEWTWWTPQEILRFMRENAGSINARVIAPESFQYLKNLSDPILNDPQALANMDILGTHLYGTQVSQFPYPLFKQKGAGKDLWMTEVYYPNSDTNSADRWPEALDVSQHIHNAMVEGDFQAYVWWYIRRSYGPMKEDGTISKRGYNMAHFSKFVRPGYVRIDATKNPNANVYVSAYKGDNKVVIVAINKSNTGVNQNFVLQNGSASNVSRWITSSSSNLQPGTNLTVSGNHFWAHLPAQSVTTFVVNR

SEQ ID NO: 8 - protein, 557 aa, Chrysobacterium sp.
MHHHHHHDEKNLLEDPDSNLSAGASARALAATPMLHVGGRYLKDPCDNNVVLHGVAITPSPWFNGCQYGANSGYCTWDNYNVQGALNYNKAVMNKLTSAADGWYLNYIRLHIDPYWTNDPGPAIPENDISRFNYNRLVTYTDQVIIPLINHARSLGMYVILRPPGVCPNRIAVNDAYHSYLKTVWTFLSQHPGLKNADNVMFELANEPVEILGTNGTWGSTGNEHFAALKNFFQPLVNIIRNNGANNVCWIPGTGWQSHYQGYVNNQITGGNIGYAVHIYPAYWGGLSNYQAFQNAWNINVKPIADIAPIAITETDWAPQGYGTFGIGTTGTAGGSGFGANLKYIVDQSGNVSWNVLAPDNLLHKGDPNAGTAYNNDWEACAAPVKQWFQQYASSNYPVGNCNTTSSLVNNGIYEIEFQTDANKVVDLKSGEDANGAVLRPWTRNGAAAQRWVAIDAGNGYWRFVSKASATNRCIDLASNSNTLGTSIRLWQNYGNDAQAWQVVAVSNGYYKILSKVDPTRGWDIPNCTMDGNSNLHLWDYYGTSCQLFKFKYIGMN

SEQ ID NO: 9 - DNA, 2731 bp, Sphingobacterium sp.
  CDS (501)..(2231)
tgactatggcttggaaggcagtggcaacaaatgtaaagggctcatcgcctatgtcggctacatcgaaggcaaaggggccaaagtggatggaatcggcacccagatgcacatcgatatcaataccagtaaagaccaaatcgtcagcatgttcaatctattggccgcaacaggcaagctgattaaagtgtctgagctcgatatcggccttggaagcggcataaagaccagcaatgcaacagctgaaatgtatcagaaacaggctgatttatacaagtttgtcgttgagaaatacctcgagatcattcccaaggataaacagtacggtatcaccctatggagcccgttggatagtccagaccaggagggttcattctggcgacgtggagagcccatcggcttatggaccgaaggatttgtccgaaagccagcctatcaggctgttgctgaggcattgtcagctaaaaaataagatcattaatcaccctttaaatatgtaaattatgagaacaaacaacatgtggttattgctgatctttttattagctattttttccagctgctcgcggctggaagaaaaaacattgaccagcgaatccgaaagaagtcttaaatccaatgtttccgcgcaagccgttacaagctggccgcggccaaccccgaccctacatgtcggaggcaagtacctcaaagatccctgcgacaataatattgtcctgcatggggtagccattacgccaagcccttggttcaatggctgtcagtatggagccaactcgggctactgcacctgggacaattacaatgtgcagggcgcgctcaattacaacaaggcggtcatggacaagctcagcagcgccgccgacggttggtacctcaattatatccgtctgcatattgatccttattggaccaatgatccaggtgcacccattcccgaagacgatatctcacggttcaactacaatcggctggttacctacaccgaccaggtcattgtccccttaatcaatcatgcccgcagccgcggtatgtatgtcatcttgcgtcctccaggtgtatgtccgcaccgtatcgccgtcaatgatgcctatcatacctatctcaagaccgtatggacctttctgtcgcagcacactgccctgaaaaatgcagacaatgtgatgtttgaattggctaacgagcctgttgaaatccttgggacgaacggtacttggggaatgacgggaaatgaacattttgctgcgctgaaaaatttctttcagcccttagtcaatatcatccgtaacaacggtgccaacaacgtctgctggatacccggtaccggttggcaatcccattaccagggttatgtcactaatcagattaccggcggaaatatcggctacgccgtacatatctatccgggttattggggcggtgtcaatacctatcaagctttccaaaatgcctggaataccaatgtcaaacctattgctgacattgcgccaatcgctattacagagaccgactgggctccacagggatatggtactttcggcacaggatctacgggcaccgctggtggtaatggttttggtgcaaatttgaaatatatcgtcgatcagtctggcaatgtcagctggaacctccttactcccgatgacctgctccataaaggggaccccaatgccggcaccgcctttaataacgattgggaggcctgcgctgcaccgagcaaacaatggtttcagcaatatgccgcctacaattaccccatgtctaactgcaccgtcaccagcttggtgaacaatgggatttacgaaattgaatttcagaccgatgccaacaaagtccttgatttgaaatcaggggaagatgccaacggtgcagcactcagaccctggacccgaaatggtgcaaacgcacagcgctgggtagccatcgatgcaggcaatggttactggcgctttgtctccaaagcaagcgcaagcagtcgttgcatcgatctgacaagtaacagtaatgtactcggaactgcgatccggctctggcagaactatggcaatgatgcgcaggcctggaaggttacagctgtagctaatggctattacaaaattacctcaaaggtagatgccacacgcggttgggatgtacccagctgcacgatggatggcaactccaatctgcagctttgggattactatggtacatcctgtcagttgtttaaattcaaatttatagcgatgaactaaaggtcatcttttcgcggtaagctattcttaccgcgaaatagtttattttaatcacatgaaaaacttcaccatgcgacaaacacaatttaaaatcctgttaatgatcttcctactatgcggtttttcaggtacagcagcgttcgcccaagacaaaaacttccatatttacctttgctttggacaatccaatatggaagggcacggtaaattcgaacctcaggataccatggccatcgaacggttcaaggtactatcggcagtagattgccccgatttagggcggcaatatggccgatggtcgccggcccgggcaccgctcacacgctgccacaccggacttacacctgcagattattttagccgaacacttgtagaaaatcttcccaaaaatattgaggtcggtgtcatcaacgtttcagtaggtggctgtcatattcaattatttgatcaggacagcacagcaagttatgttgcaaagtcaccggaatggatgaaatcca

SEQ ID NO: 10 - protein, 576 aa, Sphingobacterium sp.
MRTNNMWLLLIFLLAIFSSCSRLEEKTLTSESERSLKSNVSAQAVTSWPRPTPTLHVGGKYLKDPCDNNIVLHGVAITPSPWFNGCQYGANSGYCTWDNYNVQGALNYNKAVMDKLSSAADGWYLNYIRLHIDPYWTNDPGAPIPEDDISRFNYNRLVTYTDQVIVPLINHARSRGMYVILRPPGVCPHRIAVNDAYHTYLKTVWTFLSQHTALKNADNVMFELANEPVEILGTNGTWGMTGNEHFAALKNFFQPLVNIIRNNGANNVCWIPGTGWQSHYQGYVTNQITGGNIGYAVHIYPGYWGGVNTYQAFQNAWNTNVKPIADIAPIAITETDWAPQGYGTFGTGSTGTAGGNGFGANLKYIVDQSGNVSWNLLTPDDLLHKGDPNAGTAFNNDWEACAAPSKQWFQQYAAYNYPMSNCTVTSLVNNGIYEIEFQTDANKVLDLKSGEDANGAALRPWTRNGANAQRWVAIDAGNGYWRFVSKASASSRCIDLTSNSNVLGTAIRLWQNYGNDAQAWKVTAVANGYYKITSKVDATRGWDVPSCTMDGNSNLQLWDYYGTSCQLFKFKFIAMN

SEQ ID NO: 11 - DNA, 1698 bp, Bacillus hemicellulosilyticus
  CDS (1)..(1698)
atgcgcgaggtaggtcgcatgacgaaaatgcttcttgttgttatgttcatcgttccgcttcttctttctggccattctgcggaggcttggactggaatgcctatggacaaacttcatgtaagcggcaaccaacttgtaaacagctctggccaaactgtacttcttaacggctggcaccaaccttctggctcttactggacttaccagggctcaaactactatcttgaccgcaacggtggcaaccgccatgccgctaaccttgagtatcttaaagacatcagcgacactttcactgacacatctccgaaatacggcaacgaccacggctggtacatgaaccaaatccgccttttcatcgaccgcgaggacatgggcgacgtagcggctggcacgtataacttcgctggccttcaagaggttacgcaaaacgttatcatcccatacgttgagtacgctaaaacaaaaggcctttatgttactcttggtcttgacttcacgcttcttaacgaccaggctactactcaatctaacttagacaagttcaacgagatctggggctatcttgcttcacgtccggagcttcgcagcgctgaccacgttatgtttgagatcgtaaacgagcctgtactttcatacgcaaacggtaaatggggtggccatccatctgacccagacttcgttgaccactggaacgctcttcgcgacttccagaactctatcatcgcaacaatccgcaaccaaggcgctgacaacgttatctgggcagctggccttggctgggaccaatactaccaactttgcgcatctcacccacttactgaccctcttaacaacacaggttacgcagtacactggtatcctggctatggcgcaaacgacgactatgctactcttcaacaacaatgggacacaaacatcaaaccgtgcgcagaccattaccctatcaacatcactgagacgacttggtacaaatggcaaccaggcgacccggagtactggcacctttttgacggaacgaacgagggcttcggcaagaacacaaaagcgatctttacggacgctggcaacgtatctatcgcggttcatatgaacggcttccttcttgagcctggcgtacgctcaactttcgcggaccctactgcaggccttaagtacgacggcgatccggctcgcgacgcgatggctcgcttcatcttcgagtggtactatgaacgcgcacaactttacccgtggaacggcatctggaacggcatccacaatggcgctacttacaaacttcagaatcgcgcatctggcaaaatgatcgacgttcctggtggccaaaacaacaacggccttcagcttcaacaatgggctgacaacaacgctactgcacagcaatggatcatcgacgacatgggcacgtataacaacttctatcgccttacgtcagtatcatcttcagacaacaaggtaatggacgtacgcaacggttcttctcacaacggtgaggcgatccaacttatgtctgactttggcaactcagcgcaacaattccgccttatccgcctttctaacggctactggagcatccttaacgttaactcaaacaaggctgttgaggttacaggctcttcatctgccgatggcgctcttcttcagcaaaacatgtatcgtggcgaccttcaccaacagtgggaccttatccgcatcaactaa

SEQ ID NO: 12 - protein, 565 aa, Bacillus hemicellulosilyticus
MREVGRMTKMLLVVMFIVPLLLSGHSAEAWTGMPMDKLHVSGNQLVNSSGQTVLLNGWHQPSGSYWTYQGSNYYLDRNGGNRHAANLEYLKDISDTFTDTSPKYGNDHGWYMNQIRLFIDREDMGDVAAGTYNFAGLQEVTQNVIIPYVEYAKTKGLYVTLGLDFTLLNDQATTQSNLDKFNEIWGYLASRPELRSADHVMFEIVNEPVLSYANGKWGGHPSDPDFVDHWNALRDFQNSIIATIRNQGADNVIWAAGLGWDQYYQLCASHPLTDPLNNTGYAVHWYPGYGANDDYATLQQQWDTNIKPCADHYPINITETTWYKWQPGDPEYWHLFDGTNEGFGKNTKAIFTDAGNVSIAVHMNGFLLEPGVRSTFADPTAGLKYDGDPARDAMARFIFEWYYERAQLYPWNGIWNGIHNGATYKLQNRASGKMIDVPGGQNNNGLQLQQWADNNATAQQWIIDDMGTYNNFYRLTSVSSSDNKVMDVRNGSSHNGEAIQLMSDFGNSAQQFRLIRLSNGYWSILNVNSNKAVEVTGSSSADGALLQQNMYRGDLHQQWDLIRIN